European Patent Application EP 4 527 855 A2, published March 26, 2025. Title: STABLE IGG4 BASED BINDING AGENT FORMULATIONS. Applicant: SANOFI. Application EP. The sequence listing filed with the application follows.

SEQUENCE LISTING (29 sequences)

SEQ ID NO: 1 - protein, 5 aa, synthetic construct
GYNWH

SEQ ID NO: 2 - protein, 16 aa, synthetic construct
EITHSGSTNYNPSLKS

SEQ ID NO: 3 - protein, 14 aa, synthetic construct
EIAVAGTGYYGMDV

SEQ ID NO: 4 - protein, 11 aa, synthetic construct
RASQGINSAFA

SEQ ID NO: 5 - protein, 7 aa, synthetic construct
DASSLES

SEQ ID NO: 6 - protein, 9 aa, synthetic construct
QQFNSYPLT

SEQ ID NO: 7 - protein, 448 aa, synthetic construct
QVQLQQWGAGLLKPSETLSLTCAVYGGSFSGYNWHWIRQPPGKGLEWIGEITHSGSTNYNPSLKSRVTISVDTSKNQFSLKLSSVTAADTAVYYCVREIAVAGTGYYGMDVWGQGTTVTVSSASTKGPSVFPLAPCSRSTSESTAALGCLVKDYFPEPVTVSWNSGALTSGVHTFPAVLQSSGLYSLSSVVTVPSSSLGTKTYTCNVDHKPSNTKVDKRVESKYGPPCPPCPAPEFEGGPSVFLFPPKPKDTLMISRTPEVTCVVVDVSQEDPEVQFNWYVDGVEVHNAKTKPREEQFNSTYRVVSVLTVLHQDWLNGKEYKCKVSNKGLPSSIEKTISKAKGQPREPQVYTLPPSQEEMTKNQVSLTCLVKGFYPSDIAVEWESNGQPENNYKTTPPVLDSDGSFFLYSRLTVDKSRWQEGNVFSCSVMHEALHNHYTQKSLSLSLG

SEQ ID NO: 8 - protein, 214 aa, synthetic construct
AIQLTQSPSSLSASVGDRVTITCRASQGINSAFAWYQQKPGKAPKLLIYDASSLESGVPSRFSGSGSGTDFTLTISSLQPEDFATYYCQQFNSYPLTFGGGTKVEIKRTVAAPSVFIFPPSDEQLKSGTASVVCLLNNFYPREAKVQWKVDNALQSGNSQESVTEQDSKDSTYSLSSTLTLSKADYEKHKVYACEVTHQGLSSPVTKSFNRGEC

SEQ ID NO: 9 - protein, 240 aa, Homo sapiens
MEESVVRPSVFVVDGQTDIPFTRLGRSHRRQSCSVARVGLGLLLLLMGAGLAVQGWFLLQLHWRLGEMVTRLPDGPAGSWEQLTQERRSHEVNPAAHLTGANSSLTGSGGPLLWETQLGLAFLRGLSYHDGALVVTKAGYYYIYSKVQLGGVGCPLGLASTITHGLYKRTPRYPEELELLVSQQSPCGRATSSSRVWWDSSFLGGVVHLEAGEEVVVRVLDERLVRLRDGTRSYFGAFMV

SEQ ID NO: 10 - protein, 467 aa, synthetic construct
MKHLWFFLLLVAAPRWVLSQVQLQQWGAGLLKPSETLSLTCAVYGGSFSGYNWHWIRQPPGKGLEWIGEITHSGSTNYNPSLKSRVTISVDTSKNQFSLKLSSVTAADTAVYYCVREIAVAGTGYYGMDVWGQGTTVTVSSASTKGPSVFPLAPCSRSTSESTAALGCLVKDYFPEPVTVSWNSGALTSGVHTFPAVLQSSGLYSLSSVVTVPSSSLGTKTYTCNVDHKPSNTKVDKRVESKYGPPCPPCPAPEFEGGPSVFLFPPKPKDTLMISRTPEVTCVVVDVSQEDPEVQFNWYVDGVEVHNAKTKPREEQFNSTYRVVSVLTVLHQDWLNGKEYKCKVSNKGLPSSIEKTISKAKGQPREPQVYTLPPSQEEMTKNQVSLTCLVKGFYPSDIAVEWESNGQPENNYKTTPPVLDSDGSFFLYSRLTVDKSRWQEGNVFSCSVMHEALHNHYTQKSLSLSLG

SEQ ID NO: 11 - DNA, 1404 bp, synthetic construct
  source 1..1404: mol_type = other DNA
  CDS 1..1401
atgaagcacctgtggttctttctgctgctggtggccgctcctagatgggtgctgtcccaggtgcagctgcagcagtggggcgctggcctgctgaagccttccgagacactgtccctgacctgcgccgtgtacggcggctccttctccggctacaactggcactggatcaggcagcctcccggcaagggcctggaatggatcggcgagatcacccactccggctccaccaactacaaccctagcctgaagtccagagtgaccatctccgtggacacctccaagaaccagttctccctgaagctgtcctctgtgaccgccgctgacaccgccgtgtactactgtgtgcgggagatcgccgtggctggcaccggctactacggcatggatgtgtggggccagggcaccaccgtgaccgtgtccagcgcttctaccaagggcccttccgtgttccctctggccccttgctcccggtccacctccgagtccaccgccgctctgggctgcctggtgaaggactacttccctgagcctgtgaccgtgtcctggaactctggcgccctgacctccggcgtgcacaccttccctgccgtgctgcagtcctccggcctgtactccctgtcctccgtggtgaccgtgccttcctcctccctgggcaccaagacctacacctgtaacgtggaccacaagccttccaacaccaaggtggacaagcgggtggagtccaagtacggccctccttgccctccctgccctgcccctgagttcgagggcggacctagcgtgttcctgttccctcctaagcctaaggacaccctgatgatctcccggacccctgaggtgacctgtgtggtggtggacgtgtcccaggaggaccctgaggtccagttcaactggtacgtggacggcgtggaggtgcacaacgccaagaccaagcctcgggaggagcagttcaattccacctaccgggtggtgtctgtgctgaccgtgctgcaccaggactggctgaacggcaaagaatacaagtgtaaggtctccaacaagggcctgccctcctccatcgagaaaaccatctccaaggccaagggccagcctagggagcctcaggtgtacaccctgcctcctagccaggaagagatgaccaagaaccaggtgtccctgacctgtctggtgaagggcttctacccttccgacatcgccgtggagtgggagtccaacggccagcctgagaacaactacaagaccacccctcctgtgctggactccgacggctccttcttcctgtactccaggctgaccgtggacaagtcccggtggcaggagggcaacgtcttttcctgctccgtgatgcacgaggccctgcacaaccactacacccagaagtccctgtccctgtctctgggctga

SEQ ID NO: 12 - protein, 236 aa, synthetic construct
MDMRVPAQLLGLLLLWLPGARCAIQLTQSPSSLSASVGDRVTITCRASQGINSAFAWYQQKPGKAPKLLIYDASSLESGVPSRFSGSGSGTDFTLTISSLQPEDFATYYCQQFNSYPLTFGGGTKVEIKRTVAAPSVFIFPPSDEQLKSGTASVVCLLNNFYPREAKVQWKVDNALQSGNSQESVTEQDSKDSTYSLSSTLTLSKADYEKHKVYACEVTHQGLSSPVTKSFNRGEC

SEQ ID NO: 13 - DNA, 711 bp, synthetic construct
  source 1..711: mol_type = other DNA
  CDS 1..708
atggacatgagagtgcctgctcagctgctgggactgctgctgctgtggctgcctggcgctagatgcgccatccagctgacccagtccccctcctctctgtccgcctccgtgggcgacagagtgaccatcacctgtcgggcctcccagggcatcaactccgccttcgcctggtatcagcagaagcctggcaaggcccctaagctgctgatctacgacgcctcctccctggaatccggcgtgccctccagattttccggctccggctctggcaccgacttcaccctgaccatctccagcctgcagcctgaggacttcgccacctactactgccagcagttcaactcctaccctctgaccttcggcggaggcaccaaggtggagatcaagcgtacggtggctgcaccatctgtcttcatcttcccgccatctgatgagcagttgaaatctggaactgcctctgttgtgtgcctgctgaataacttctatcccagagaggccaaagtacagtggaaggtggataacgccctccaatcgggtaactcccaggagagtgtcacagagcaggacagcaaggacagcacctacagcctcagcagcaccctgacgctgagcaaagcagactacgagaaacacaaagtctacgcctgcgaagtcacccatcagggcctgagctcgcccgtcacaaagagcttcaacaggggagagtgttag

SEQ ID NO: 14 - protein, 372 aa, Homo sapiens
MNYPLTLEMDLENLEDLFWELDRLDNYNDTSLVENHLCPATEGPLMASFKAVFVPVAYSLIFLLGVIGNVLVLVILERHRQTRSSTETFLFHLAVADLLLVFILPFAVAEGSVGWVLGTFLCKTVIALHKVNFYCSSLLLACIAVDRYLAIVHAVHAYRHRRLLSIHITCGTIWLVGFLLALPEILFAKVSQGHHNNSLPRCTFSQENQAETHAWFTSRFLYHVAGFLLPMLVMGWCYVGVVHRLRQAQRRPQRQKAVRVAILVTSIFFLCWSPYHIVIFLDTLARLKAVDNTCKLNGSLPVAITMCEFLGLAHCCLNPMLYTFAGVKFRSDLSRLLTKLGCTGPASLCQLFPSWRRSSLSESENATSLTTF

SEQ ID NO: 15 - protein, 10 aa, synthetic construct
GFSLIDYGVN

SEQ ID NO: 16 - protein, 9 aa, synthetic construct
VIWGDGTTY

SEQ ID NO: 17 - skipped

SEQ ID NO: 18 - protein, 16 aa, synthetic construct
RSSKSLLHSSGKTYLY

SEQ ID NO: 19 - protein, 6 aa, synthetic construct
RLSSLA

SEQ ID NO: 20 - protein, 9 aa, synthetic construct
MQHLEYPYT

SEQ ID NO: 21 - protein, 111 aa, synthetic construct
QVQLKESGPGLVAPSESLSITCTVSGFSLIDYGVNWIRQPPGKGLEWLGVIWGDGTTYYNPSLKSRLSISKDNSKSQVFLKVTSLTTDDTAMYYCARIVYWGQGTLVTVSA

SEQ ID NO: 22 - protein, 112 aa, synthetic construct
DIVMTQAAPSVAVTPGASVSISCRSSKSLLHSSGKTYLYWFLQRPGQSPQLLIYRLSSLASGVPDRFSGSGSGTAFTLRISRVEAEDVGVYYCMQHLEYPYTFGGGTKLEIK

SEQ ID NO: 23 - protein, 326 aa, synthetic construct
ASTKGPSVFPLAPCSRSTSESTAALGCLVKDYFPEPVTVSWNSGALTSGVHTFPAVLQSSGLYSLSSVVTVPSSSLGTKTYTCNVDHKPSNTKVDKRVESKYGPPCPPCPAPEFEGGPSVFLFPPKPKDTLMISRTPEVTCVVVDVSQEDPEVQFNWYVDGVEVHNAKTKPREEQFNSTYRVVSVLTVLHQDWLNGKEYKCKVSNKGLPSSIEKTISKAKGQPREPQVYTLPPSQEEMTKNQVSLTCLVKGFYPSDIAVEWESNGQPENNYKTTPPVLDSDGSFFLYSRLTVDKSRWQEGNVFSCSVMHEALHNHYTQKSLSLSLG

SEQ ID NO: 24 - protein, 107 aa, synthetic construct [sequence omitted]

SEQ ID NO: 25 - protein, 437 aa, synthetic construct
QVQLKESGPGLVAPSESLSITCTVSGFSLIDYGVNWIRQPPGKGLEWLGVIWGDGTTYYNPSLKSRLSISKDNSKSQVFLKVTSLTTDDTAMYYCARIVYWGQGTLVTVSAASTKGPSVFPLAPCSRSTSESTAALGCLVKDYFPEPVTVSWNSGALTSGVHTFPAVLQSSGLYSLSSVVTVPSSSLGTKTYTCNVDHKPSNTKVDKRVESKYGPPCPPCPAPEFEGGPSVFLFPPKPKDTLMISRTPEVTCVVVDVSQEDPEVQFNWYVDGVEVHNAKTKPREEQFNSTYRVVSVLTVLHQDWLNGKEYKCKVSNKGLPSSIEKTISKAKGQPREPQVYTLPPSQEEMTKNQVSLTCLVKGFYPSDIAVEWESNGQPENNYKTTPPVLDSDGSFFLYSRLTVDKSRWQEGNVFSCSVMHEALHNHYTQKSLSLSLG

SEQ ID NO: 26 - protein, 219 aa, synthetic construct
  REGION 1..219: note = source = /note="Description of Artificial Sequence: Synthetic polypeptide"
DIVMTQAAPSVAVTPGASVSISCRSSKSLLHSSGKTYLYWFLQRPGQSPQLLIYRLSSLASGVPDRFSGSGSGTAFTLRISRVEAEDVGVYYCMQHLEYPYTFGGGTKLEIKRTVAAPSVFIFPPSDEQLKSGTASVVCLLNNFYPREAKVQWKVDNALQSGNSQESVTEQDSKDSTYSLSSTLTLSKADYEKHKVYACEVTHQGLSSPVTKSFNRGEC

SEQ ID NO: 27 - protein, 19 aa, synthetic construct
MGWSCIILFLVATATGVHS

SEQ ID NO: 28 - protein, 456 aa, synthetic construct
MGWSCIILFLVATATGVHSQVQLKESGPGLVAPSESLSITCTVSGFSLIDYGVNWIRQPPGKGLEWLGVIWGDGTTYYNPSLKSRLSISKDNSKSQVFLKVTSLTTDDTAMYYCARIVYWGQGTLVTVSAASTKGPSVFPLAPCSRSTSESTAALGCLVKDYFPEPVTVSWNSGALTSGVHTFPAVLQSSGLYSLSSVVTVPSSSLGTKTYTCNVDHKPSNTKVDKRVESKYGPPCPPCPAPEFEGGPSVFLFPPKPKDTLMISRTPEVTCVVVDVSQEDPEVQFNWYVDGVEVHNAKTKPREEQFNSTYRVVSVLTVLHQDWLNGKEYKCKVSNKGLPSSIEKTISKAKGQPREPQVYTLPPSQEEMTKNQVSLTCLVKGFYPSDIAVEWESNGQPENNYKTTPPVLDSDGSFFLYSRLTVDKSRWQEGNVFSCSVMHEALHNHYTQKSLSLSLG

SEQ ID NO: 29 - protein, 238 aa, synthetic construct
MGWSCIILFLVATATGVHSDIVMTQAAPSVAVTPGASVSISCRSSKSLLHSSGKTYLYWFLQRPGQSPQLLIYRLSSLASGVPDRFSGSGSGTAFTLRISRVEAEDVGVYYCMQHLEYPYTFGGGTKLEIKRTVAAPSVFIFPPSDEQLKSGTASVVCLLNNFYPREAKVQWKVDNALQSGNSQESVTEQDSKDSTYSLSSTLTLSKADYEKHKVYACEVTHQGLSSPVTKSFNRGEC